European Patent Specification EP 2 953 966 B1, published March 27, 2024. Title: Induction of cross-reactive cellular response against rhinovirus antigens. Applicant: Sanofi-Pasteur Imperial Innovations Limited. The sequence listing filed with the application follows.

SEQUENCE LISTING (41 sequences)

SEQ ID NO: 1 - protein, 69 aa, Artificial Sequence
  HRV16 VP4 peptide
MGAQVSRQNVGTHSTQNMVSNGSSLNYFNINYFKDAASSGASRLDFSQDPSKFTDPVKDVLEKGIPTLQ

SEQ ID NO: 2 - protein, 69 aa, Artificial Sequence
  HRV14 VP4 peptide
MGAQVSTQKSGSHENQNILTNGSNQTFTVINYYKDAASTSSAGQSLSMDPSKFTEPVKDLMLKGAPALN

SEQ ID NO: 3 - protein, 260 aa, Artificial Sequence
  HRV16 VP2 peptide
SPSVEACGYSDRIIQITRGDSTITSQDVANAVVGYGVWPHYLTPQDATAIDKPTQPDTSSNRFYTLDSKMWNSTSKGWWWKLPDALKDMGIFGENMFYHFLGRSGYTVHVQCNASKFHQGTLLVVMIPEHQLATVNKGNVNAGYKYTHPGEAGREVGTQVENEKQPSDDNWLNFDGTLLGNLLIFPHQFINLRSNNSATLIVPYVNAVPMDSMVRHNNWSLVIIPVCQLQSNNISNIVPITVSISPMCAEFSGARAKTVV

SEQ ID NO: 4 - protein, 260 aa, Artificial Sequence
  HRV14 VP2 peptide
SPNVEACGYSDRVQQITLGNSTITTQEAANAVVCYAEWPEYLPDVDASDVNKTSKPDTSVCRFYTLDSKTWTTGSKGWCWKLPDALKDMGVFGQNMFFHSLGRSGYTVHVQCNATKFHSGCLLVVVIPEHQLASHEGGNVSVKYTFTHPGERGIDLSSANEVGGPVKDVIYNMNGTLLGNLLIFPHQFINLRTNNTATIVIPYINSVPIDSMTRHNNVSLMVIPIAPLTVPTGATPSLPITVTIAPMCTEFSGIRSKSIV

SEQ ID NO: 5 - protein, 135 aa, Artificial Sequence
  HRV16 VP135
MGAQVSRQNVGTHSTQNMVSNGSSLNYFNINYFKDAASSGASRLDFSQDPSKFTDPVKDVLEKGIPTLQSPSVEACGYSDRIIQITRGDSTITSQDVANAVVGYGVWPHYLTPQDATAIDKPTQPDTSSNRFYTL

SEQ ID NO: 6 - protein, 329 aa, Artificial Sequence
  HRV16 VP0 polyprotein
MGAQVSRQNVGTHSTQNMVSNGSSLNYFNINYFKDAASSGASRLDFSQDPSKFTDPVKDVLEKGIPTLQSPSVEACGYSDRIIQITRGDSTITSQDVANAVVGYGVWPHYLTPQDATAIDKPTQPDTSSNRFYTLDSKMWNSTSKGWWWKLPDALKDMGIFGENMFYHFLGRSGYTVHVQCNASKFHQGTLLVVMIPEHQLATVNKGNVNAGYKYTHPGEAGREVGTQVENEKQPSDDNWLNFDGTLLGNLLIFPHQFINLRSNNSATLIVPYVNAVPMDSMVRHNNWSLVIIPVCQLQSNNISNIVPITVSISPMCAEFSGARAKTVV

SEQ ID NO: 7 - protein, 135 aa, Artificial Sequence
  HRV14 VP135
MGAQVSTQKSGSHENQNILTNGSNQTFTVINYYKDAASTSSAGQSLSMDPSKFTEPVKDLMLKGAPALNSPNVEACGYSDRVQQITLGNSTITTQEAANAVVCYAEWPEYLPDVDASDVNKTSKPDTSVCRFYTL

SEQ ID NO: 8 - protein, 329 aa, Artificial Sequence
  HRV14 VP0 polyprotein
  SITE (1)..(171): pool E
MGAQVSTQKSGSHENQNILTNGSNQTFTVINYYKDAASTSSAGQSLSMDPSKFTEPVKDLMLKGAPALNSPNVEACGYSDRVQQITLGNSTITTQEAANAVVCYAEWPEYLPDVDASDVNKTSKPDTSVCRFYTLDSKTWTTGSKGWCWKLPDALKDMGVFGQNMFFHSLGRSGYTVHVQCNATKFHSGCLLVVVIPEHQLASHEGGNVSVKYTFTHPGERGIDLSSANEVGGPVKDVIYNMNGTLLGNLLIFPHQFINLRTNNTATIVIPYINSVPIDSMTRHNNVSLMVIPIAPLTVPTGATPSLPITVTIAPMCTEFSGIRSKSIV

SEQ ID NO: 9 - protein, 105 aa, Artificial Sequence
  last 105 amino acids of HRV16 RNA polymerase
ADKSSEFKELDYGNVTFLKRGFRQDDKYKFLIHPTFPVEEIYESIRWTKKPSQMQEHVLSLCHLMWHNGPEIYKDFETKIRSVSAGRALYIPPYELLRHEWYEKF

SEQ ID NO: 10 - protein, 105 aa, Artificial Sequence
  last 105 amino acids of HRV14 RNA polymerase
PDKSETFTKMTWENLTFLKRYFKPDQQFPFLVHPVMPMKDIHESIRWTKDPKNTQDHVRSLCMLAWHSGEKEYNEFIQKIRTTDIGKCLILPEYSVLRRRWLDLF

SEQ ID NO: 11 - protein, 240 aa, Artificial Sequence
  HRV16 VP-pol fusion peptide
MGAQVSRQNVGTHSTQNMVSNGSSLNYFNINYFKDAASSGASRLDFSQDPSKFTDPVKDVLEKGIPTLQSPSVEACGYSDRIIQITRGDSTITSQDVANAVVGYGVWPHYLTPQDATAIDKPTQPDTSSNRFYTLADKSSEFKELDYGNVTFLKRGFRQDDKYKFLIHPTFPVEEIYESIRWTKKPSQMQEHVLSLCHLMWHNGPEIYKDFETKIRSVSAGRALYIPPYELLRHEWYEKF

SEQ ID NO: 12 - protein, 240 aa, Artificial Sequence
  HRV14 VP-Pol fusion peptide
MGAQVSTQKSGSHENQNILTNGSNQTFTVINYYKDAASTSSAGQSLSMDPSKFTEPVKDLMLKGAPALNSPNVEACGYSDRVQQITLGNSTITTQEAANAVVCYAEWPEYLPDVDASDVNKTSKPDTSVCRFYTLPDKSETFTKMTWENLTFLKRYFKPDQQFPFLVHPVMPMKDIHESIRWTKDPKNTQDHVRSLCMLAWHSGEKEYNEFIQKIRTTDIGKCLILPEYSVLRRRWLDLF

SEQ ID NO: 13 - protein, 363 aa, Artificial Sequence
  C-ter domain of HRV16 RNA polymerase
EDSVFGMDGLEALDLNTSAGYPYVTLGIKKKDLINNKTKDISKLKLALDKYDVDLPMITFLKDELRKKDKIAAGKTRVIEASSINDTILFRTVYGNLFSKFHLNPGVVTGCAVGCDPETFWSKIPLMLDGDCIMAFDYTNYDGSIHPIWFKALGMVLDNLSFNPTLINRLCNSKHIFKSTYYEVEGGVPSGCSGTSIFNSMINNIIIRTLVLDAYKHIDLDKLKIIAYGDDVIFSYKYKLDMEAIAKEGQKYGLTITPADKSSEFKELDYGNVTFLKRGFRQDDKYKFLIHPTFPVEEIYESIRWTKKPSQMQEHVLSLCHLMWHNGPEIYKDFETKIRSVSAGRALYIPPYELLRHEWYEKF

SEQ ID NO: 14 - protein, 363 aa, Artificial Sequence
  C-terminal domain of HRV14 RNA polymerase
  SITE (186)..(363): Pool F
KEALYGVDGLEPIDITTSAGFPYVSLGIKKRDILNKETQDTEKMKFYLDKYGIDLPLVTYIKDELRSVDKVRLGKSRLIEASSLNDSVNMRMKLGNLYKAFHQNPGVLTGSAVGCDPDVFWSVIPCLMDGHLMAFDYSNFDASLSPVWFVCLEKVLTKLGFAGSSLIQSICNTHHIFRDEIYVVEGGMPSGCSGTSIFNSMINNIIIRTLILDAYKGIDLDKLKILAYGDDLIVSYPYELDPQVLATLGKNYGLTITPPDKSETFTKMTWENLTFLKRYFKPDQQFPFLVHPVMPMKDIHESIRWTKDPKNTQDHVRSLCMLAWHSGEKEYNEFIQKIRTTDIGKCLILPEYSVLRRRWLDLF

SEQ ID NO: 15 - protein, 460 aa, Artificial Sequence
  HRV16 RNA polymerase
GQIQISKHVKDVGLPSIHTPTKTKLQPSVFYDIFPGSKEPAVLTEKDPRLKVDFDSALFSKYKGNTECSLNEHIQVAVAHYSAQLATLDIDPQPIAMEDSVFGMDGLEALDLNTSAGYPYVTLGIKKKDLINNKTKDISKLKLALDKYDVDLPMITFLKDELRKKDKIAAGKTRVIEASSINDTILFRTVYGNLFSKFHLNPGVVTGCAVGCDPETFWSKIPLMLDGDCIMAFDYTNYDGSIHPIWFKALGMVLDNLSFNPTLINRLCNSKHIFKSTYYEVEGGVPSGCSGTSIFNSMINNIIIRTLVLDAYKHIDLDKLKIIAYGDDVIFSYKYKLDMEAIAKEGQKYGLTITPADKSSEFKELDYGNVTFLKRGFRQDDKYKFLIHPTFPVEEIYESIRWTKKPSQMQEHVLSLCHLMWHNGPEIYKDFETKIRSVSAGRALYIPPYELLRHEWYEKF

SEQ ID NO: 16 - protein, 460 aa, Artificial Sequence
  HRV14 RNA polymerase
GQVIARHKVREFNINPVNTPTKSKLHPSVFYDVFPGDKEPAVLSDNDPRLEVKLTESLFSKYKGNVNTEPTENMLVAVDHYAGQLLSLDIPTSELTLKEALYGVDGLEPIDITTSAGFPYVSLGIKKRDILNKETQDTEKMKFYLDKYGIDLPLVTYIKDELRSVDKVRLGKSRLIEASSLNDSVNMRMKLGNLYKAFHQNPGVLTGSAVGCDPDVFWSVIPCLMDGHLMAFDYSNFDASLSPVWFVCLEKVLTKLGFAGSSLIQSICNTHHIFRDEIYVVEGGMPSGCSGTSIFNSMINNIIIRTLILDAYKGIDLDKLKILAYGDDLIVSYPYELDPQVLATLGKNYGLTITPPDKSETFTKMTWENLTFLKRYFKPDQQFPFLVHPVMPMKDIHESIRWTKDPKNTQDHVRSLCMLAWHSGEKEYNEFIQKIRTTDIGKCLILPEYSVLRRRWLDLF

SEQ ID NO: 17 - protein, 332 aa, Artificial Sequence
  HRV1B VP0 polyprotein
  SITE (1)..(171): Pool C
  SITE (172)..(332): Pool D
MGAQVSRQNVGTHSTQNSVSNGSSLNYFNINYFKDAASSGASRLDFSQDPSKFTDPVKDVLEKGIPTLQSPSVEACGYSDRIIQITRGDSTITSQDVANAVVGYGVWPHYLTPQDATAIDKPTQPDTSSNRFYTLESKHWNGDSKGWWWKLPDALKEMGIFGENMYYHFLGRSGYTVHVQCNASKFHQGTLLVAMIPEHQLASAKNGSVTAGYNLTHPGEAGRVVGQQRDANLRQPSDDSWLNFDGTLLGNLLIFPHQFINLRSNNSATLIVPYVNAVPMDSMLRHNNWSLVIIPISPLRSETTSSNIRPITVSISPMCAEFSGARAKNVRQ

SEQ ID NO: 18 - protein, 365 aa, Artificial Sequence
  HRV1B RNA polymerase
  SITE (1)..(187): Pool A
  SITE (188)..(365): Pool B
MLEDSVFGIEGLEALDLNTSAGFPYVTMGIKKRDLINNKTKDISRLKEALDKYGVDLPMITFLKDELRKKEKISAGKTRVIEASSINDTILFRTTFGNLFSKFHLNPGVVTGSAVGCDPETFWSKIPVMLDGDCIMAFDYTNYDGSIHPVWFQALKKVLENLSFQSNLIDRLCYSKHLFKSTYYEVAGGVPSGCSGTSIFNTMINNIIIRTLVLDAYKNIDLDKLKIIAYGDDVIFSYKYTLDMEAIANEGKKYGLTITPADKSTEFKKLDYNNVTFLKRGFKQDEKHTFLIHPTFPVEEIYESIRWTKKPSQMQEHVLSLCHLMWHNGRKVYEDFSSKIRSVSAGRALYIPPYDLLKHEWYEKF

SEQ ID NO: 19 - protein, 239 aa, Artificial Sequence
  HRV1 VP-Pol fusion protein
GAQVSRQNVGTHSTQNSVSNGSSLNYFNINYFKDAASSGASRLDFSQDPSKFTDPVKDVLEKGIPTLQSPSVEACGYSDRIIQITRGDSTITSQDVANAVVGYGVWPHYLTPQDATAIDKPTQPDTSSNRFYTLADKSTEFKKLDYNNVTFLKRGFKQDEKHTFLIHPTFPVEEIYESIRWTKKPSQMQEHVLSLCHLMWHNGRKVYEDFSSKIRSVSAGRALYIPPYDLLKHEWYEKF

SEQ ID NO: 20 - protein, 331 aa, Artificial Sequence
  HRV29 VP0 polyprotein
GAQVSRQNVGTHSTQNSVSNGSSLNYFNINYFKDAASSGASKLEFSQDPSKFTDPVKDVLEKGIPTLQSPTVEACGYSDRIMQITRGDSTITSQDVANAVIGYGVWPHYLSAEDATAIDKPTQPDTSSNRFYTLESKTWDRQSKGWWWKLPDALKDMGIFGENMYYHYLGRSGYTVHVQCNASKFHQGTLLVVMILEHQLASVGTEKVGPGYNFTHPGEAGRQIGNVSDRTSKHPSDDNWLNFDGTLLGNVLIFPHQFINLRSNNSATIIVPYVNAVPMDSMLRHNNWSLVIIPISELQTENATNLTVPITVSISPMFAEFSGARARPARA

SEQ ID NO: 21 - protein, 362 aa, Artificial Sequence
  HRV29 RNA polymerase
ESVFGIEGLEALDLNTSAGFPYISMGIKKRDLINKQTKDVTKLKMALDKYGVDLPMVTFLKDELRKREKICAGKTRVIEASSVNDTILFRTTFGNLFSKFHLNPGVVTGSAVGCDPETFWSKIPVMLDGECIMAFDYTNYDGSIHPIWFQALKEVLANLSFEPALIDRLCRSKHIFKNTYYEVEGGIPSGCSGTSIFNTMINNVIIRTLVLDAYKNIDLDKLKILAYGDDVIFSYKYQLDMEAIAKEGTKYGLTITPADKSDCFKQLNYNNVTFLKRGFRQDEKHNFLIHPTFPVEEIQESIRWTKKPSQMQEHVLSLCHLMWHNGRDVYKQFEDRIRSVSAGRALYIPPYDLLLHEWYEKF

SEQ ID NO: 22 - protein, 239 aa, Artificial Sequence
  HRV29 VP-Pol fusion peptide
GAQVSRQNVGTHSTQNSVSNGSSLNYFNINYFKDAASSGASKLEFSQDPSKFTDPVKDVLEKGIPTLQSPTVEACGYSDRIMQITRGDSTITSQDVANAVIGYGVWPHYLSAEDATAIDKPTQPDTSSNRFYTLADKSDCFKQLNYNNVTFLKRGFRQDEKHNFLIHPTFPVEEIQESIRWTKKPSQMQEHVLSLCHLMWHNGRDVYKQFEDRIRSVSAGRALYIPPYDLLLHEWYEKF

SEQ ID NO: 23 - DNA, 19 bp, Artificial Sequence
  IL-4 forward primer
acaggagaagggacgccat

SEQ ID NO: 24 - DNA, 21 bp, Artificial Sequence
  IL-4 reverse primer
gaagccctacagacgagctca

SEQ ID NO: 25 - DNA, 18 bp, Artificial Sequence
  IL-4 probe
tcctcacagcaacgaaga

SEQ ID NO: 26 - DNA, 24 bp, Artificial Sequence
  IFN-g forward primer
tcaagtggcatagatgtggaagaa

SEQ ID NO: 27 - DNA, 21 bp, Artificial Sequence
  IFN-g reverse primer
tggctctgcaggattttcatg

SEQ ID NO: 28 - DNA, 20 bp, Artificial Sequence
  IFN-g probe
tcaccatccttttgccagtt

SEQ ID NO: 29 - DNA, 22 bp, Artificial Sequence
  IL-17a forward primer
tcagactacctcaaccgttcca

SEQ ID NO: 30 - DNA, 21 bp, Artificial Sequence
  IL-17a reverse primer
agcttcccagatcacagaggg

SEQ ID NO: 31 - DNA, 22 bp, Artificial Sequence
  IL-17a probe
tcaccctggactctccaccgca

SEQ ID NO: 32 - DNA, 19 bp, Artificial Sequence
  HRV forward primer
gtgaagagccscrtgtgct

SEQ ID NO: 33 - DNA, 21 bp, Artificial Sequence
  HRV reverse primer
gctscagggttaaggttagcc

SEQ ID NO: 34 - DNA, 22 bp, Artificial Sequence
  HRV probe
tgagtcctccggcccctgaatg

SEQ ID NO: 35 - DNA, 21 bp, Artificial Sequence
  18S forward primer
cgccgctagaggtgaaattct

SEQ ID NO: 36 - DNA, 21 bp, Artificial Sequence
  18S reverse primer
cattcttggcaaatgctttcg

SEQ ID NO: 37 - DNA, 21 bp, Artificial Sequence
  18S probe
accggcgcaagacggaccaga

SEQ ID NO: 38 - DNA, 20 bp, Artificial Sequence
  CpG ODN 1826
tccatgacgttcctgacgtt

SEQ ID NO: 39 - DNA, 19 bp, Artificial Sequence
  CpG ODN 2216
gggggacgatcgtcggggg

SEQ ID NO: 40 - DNA, 21 bp, Artificial Sequence
  CpG 2336
ggggacgacgtcgtggggggg

SEQ ID NO: 41 - DNA, 24 bp, Artificial Sequence
  CpG 7909
tcgtcgttttgtcgttttgtcgtt